European Patent Application EP 4 481 039 A1, published December 25, 2024. Title: Novel variant of zinc-binding dehydrogenase and method for preparing L-aromatic amino acid using the same. Applicant: DAESANG CORPORATION. The sequence listing filed with the application follows.

SEQUENCE LISTING (24 sequences)

SEQ ID NO: 1 - protein, 425 aa, synthetic construct
MKTKVAAIYGKRDVRLRVFELPEITDNELLVSVISDSVCLSTWKAALLGSEHKRVPDDLENHPVITGHECAGVIVEVGKNLTGKYKKGQRFVLQPAMGLPSRYSAGYSYEYFGGNATYMIIPEIAINLGCVLPYHGSYFAAASLAEPMCCIIGAYHANYHTTQYVYEHRMGVKPGGNIALLACAGPMGIGAIDYAINGGIQPSRVVVVDIDDKRLAQVQKLLPVELAASKGIELVYVNTKGMSDPVQMLRALTGDAGFDDIFVYAAVPAVVEMADELLAEDGCLNFFAGPTDKNFKVPFNFYNVHYNSTHVVGTSGGSTDDMKEAIALSATGQLQPSFMVTHIGGLDAVPETVLNLPDIPGGKKLIYNGVTMPLTAIADFAEKGKTDPLFKELARLVEETHGIWNEQAEKYLLAQFGVDIGEAAQ

SEQ ID NO: 2 - DNA, 1278 bp, synthetic construct
  source 1..1278: mol_type = other DNA
atgaaaaccaaagttgctgctatttatggcaagcgggatgtccgtctgcgcgtatttgaactgccagaaattaccgataatgaattactggtgagtgtaatttctgacagcgtctgtttatcgacctggaaagcggcgttactcggtagtgaacataaacgcgtacccgacgatttagaaaatcatccggtcattaccgggcatgaatgtgccggggttattgtcgaagtgggtaaaaatctcactggcaaatataaaaaaggccagcgttttgtattgcaaccggcgatggggttaccaagcagatattcagcgggctacagctacgaatattttggcggcaatgccacttatatgattattcccgaaatcgccattaatttgggctgcgtattaccgtatcacggctcttattttgctgcggcgtcgctggcagagcctatgtgctgcattattggtgcttatcatgccaattatcacaccacgcaatatgtttatgagcatcgcatgggcgtcaaacctggcggcaatattgcactgctggcgtgtgcaggtccgatgggcattggcgctatcgattacgccattaacggcggcatacaaccgtcgcgggtggtggtggtcgatatcgacgacaaacgtctggcgcaggtacagaagctgctgccggtggaactggcggccagtaaaggcattgagctggtgtatgtgaataccaaagggatgagcgatcctgtccagatgctgcgggcgctgacaggagatgccgggttcgatgacatttttgtttatgcggcggtgcctgctgtcgttgagatggctgatgaattactggcggaagatggctgtctgaacttctttgccgggccgacggataaaaacttcaaagtgccgtttaatttctacaacgtccattacaacagcacgcacgtcgtcggtacatctggcggttcaacggacgacatgaaagaggcgattgcccttagcgccactgggcagttacagccgtcgtttatggtgacccatatcggtggcctggatgcggtgccagaaaccgtgctcaatctgccggatatccctggcggtaaaaaactcatttataacggcgtgaccatgccgctcactgccattgccgattttgccgaaaaaggcaaaaccgatccgctgtttaaagagttggcgcggctggttgaggaaacgcacggcatctggaatgaacaggccgagaaatatctgctggcacaatttggcgttgatatcggggaggccgcgcaatga

SEQ ID NO: 3 - protein, 425 aa, Escherichia coli
MKTKVAAIYGKRDVRLRVFELPEITDNELLVSVISDSVCLSTWKAALLGSEHKRVPDDLENHPVITGHECAGVIVEVGKNLTGKYKKGQRFVLQPAMGLPSGYSAGYSYEYFGGNATYMIIPEIAINLGCVLPYHGSYFAAASLAEPMCCIIGAYHANYHTTQYVYEHRMGVKPGGNIALLACAGPMGIGAIDYAINGGIQPSRVVVVDIDDKRLAQVQKLLPVELAASKGIELVYVNTKGMSDPVQMLRALTGDAGFDDIFVYAAVPAVVEMADELLAEDGCLNFFAGPTDKNFKVPFNFYNVHYNSTHVVGTSGGSTDDMKEAIALSATGQLQPSFMVTHIGGLDAVPETVLNLPDIPGGKKLIYNGVTMPLTAIADFAEKGKTDPLFKELARLVEETHGIWNEQAEKYLLAQFGVDIGEAAQ

SEQ ID NO: 4 - DNA, 1278 bp, Escherichia coli
  source 1..1278: mol_type = genomic DNA
atgaaaaccaaagttgctgctatttatggcaagcgggatgtccgtctgcgcgtatttgaactgccagaaattaccgataatgaattactggtgagtgtaatttctgacagcgtctgtttatcgacctggaaagcggcgttactcggtagtgaacataaacgcgtacccgacgatttagaaaatcatccggtcattaccgggcatgaatgtgccggggttattgtcgaagtgggtaaaaatctcactggcaaatataaaaaaggccagcgttttgtattgcaaccggcgatggggttaccaagcggatattcagcgggctacagctacgaatattttggcggcaatgccacttatatgattattcccgaaatcgccattaatttgggctgcgtattaccgtatcacggctcttattttgctgcggcgtcgctggcagagcctatgtgctgcattattggtgcttatcatgccaattatcacaccacgcaatatgtttatgagcatcgcatgggcgtcaaacctggcggcaatattgcactgctggcgtgtgcaggtccgatgggcattggcgctatcgattacgccattaacggcggcatacaaccgtcgcgggtggtggtggtcgatatcgacgacaaacgtctggcgcaggtacagaagctgctgccggtggaactggcggccagtaaaggcattgagctggtgtatgtgaataccaaagggatgagcgatcctgtccagatgctgcgggcgctgacaggagatgccgggttcgatgacatttttgtttatgcggcggtgcctgctgtcgttgagatggctgatgaattactggcggaagatggctgtctgaacttctttgccgggccgacggataaaaacttcaaagtgccgtttaatttctacaacgtccattacaacagcacgcacgtcgtcggtacatctggcggttcaacggacgacatgaaagaggcgattgcccttagcgccactgggcagttacagccgtcgtttatggtgacccatatcggtggcctggatgcggtgccagaaaccgtgctcaatctgccggatatccctggcggtaaaaaactcatttataacggcgtgaccatgccgctcactgccattgccgattttgccgaaaaaggcaaaaccgatccgctgtttaaagagttggcgcggctggttgaggaaacgcacggcatctggaatgaacaggccgagaaatatctgctggcacaatttggcgttgatatcggggaggccgcgcaatga

SEQ ID NO: 5 - DNA, 30 bp, synthetic construct
  source 1..30: mol_type = other DNA
caattttattatagtaattgactattatac

SEQ ID NO: 6 - DNA, 40 bp, synthetic construct
  source 1..40: mol_type = other DNA
gcttggtaaccaattttattatagtaattgactattatac

SEQ ID NO: 7 - DNA, 40 bp, synthetic construct
  source 1..40: mol_type = other DNA
gttaccaagcggatattcaggttttagagctagaaatagc

SEQ ID NO: 8 - DNA, 30 bp, synthetic construct
  source 1..30: mol_type = other DNA
ggatattcaggttttagagctagaaatagc

SEQ ID NO: 9 - DNA, 21 bp, synthetic construct
  source 1..21: mol_type = other DNA
gagcctgtcggcctacctgct

SEQ ID NO: 10 - DNA, 20 bp, synthetic construct
  source 1..20: mol_type = other DNA
cggccggcatgagcctgtcg

SEQ ID NO: 11 - DNA, 30 bp, synthetic construct
  source 1..30: mol_type = other DNA
atgccggccggctgctatttatggcaagcg

SEQ ID NO: 12 - DNA, 20 bp, synthetic construct
  source 1..20: mol_type = other DNA
gctgctatttatggcaagcg

SEQ ID NO: 13 - DNA, 20 bp, synthetic construct
  source 1..20: mol_type = other DNA
cccatcgccggttgcaatac

SEQ ID NO: 14 - DNA, 20 bp, synthetic construct
  source 1..20: mol_type = other DNA
gcttggtaaccccatcgccg

SEQ ID NO: 15 - DNA, 30 bp, synthetic construct
  source 1..30: mol_type = other DNA
gttaccaagcagatattcagcgggctacag

SEQ ID NO: 16 - DNA, 20 bp, synthetic construct
  source 1..20: mol_type = other DNA
agatattcagcgggctacag

SEQ ID NO: 17 - DNA, 20 bp, synthetic construct
  source 1..20: mol_type = other DNA
tgctcataaacatattgcgt

SEQ ID NO: 18 - DNA, 20 bp, synthetic construct
  source 1..20: mol_type = other DNA
gcccatgcgatgctcataaa

SEQ ID NO: 19 - DNA, 33 bp, synthetic construct
  source 1..33: mol_type = other DNA
tcgcatgggcgagctcctgaaaatctcgataac

SEQ ID NO: 20 - DNA, 23 bp, synthetic construct
  source 1..23: mol_type = other DNA
gagctcctgaaaatctcgataac

SEQ ID NO: 21 - DNA, 20 bp, synthetic construct
  source 1..20: mol_type = other DNA
acgtgtgacggataaaccac

SEQ ID NO: 22 - DNA, 20 bp, synthetic construct
  source 1..20: mol_type = other DNA
ttcacatacaccagctcaat

SEQ ID NO: 23 - DNA, 3234 bp, synthetic construct
  source 1..3234: mol_type = other DNA
tttccataggctccgcccccctgacgagcatcacaaaaatcgacgctcaagtcagaggtggcgaaacccgacaggactataaagataccaggcgtttccccctggaagctccctcgtgcgctctcctgttccgaccctgccgcttaccggatacctgtccgcctttctcccttcgggaagcgtggcgctttctcatagctcacgctgtaggtatctcagttcggtgtaggtcgttcgctccaagctgggctgtgtgcacgaaccccccgttcagcccgaccgctgcgccttatccggtaactatcgtcttgagtccaacccggtaagacacgacttatcgccactggcagcagccactggtaacaggattagcagagcgaggtatgtaggcggtgctacagagttcttgaagtggtggcctaactacggctacactagaaggacagtatttggtatctgcgctctgctgaagccagttaccttcggaaaaagagttggtagctcttgatccggcaaacaaaccaccgctggtagcggtggtttttttgtttgcaagcagcagattacgcgcagaaaaaaaggatctcaagaagatcctttgatcttttctacggggtctgacgctcagtggaacgaaaactcacgttaagggattttggtcatgagattatcaaaaaggatcttcacctagatccttttaaattaaaaatgaagttttaaatcaatctaaagtatatatgagtaaacttggtctgacagttaaaagattgacagtataatagtcaattactataataaaattgatgcgcaggtgaaacacctgctgcagttttagagctagaaatagcaagttaaaataaggctagtccgttatcaacttgaaaaagtggcaccgagtcggtgctttttttcgttttccgggacgccctcgcggacgtgctcatagtccacgacgcccgtgattttgtagccctggccgacggccagcaggtaggccgacaggctcatgccggccggagctcctgaaaatctcgataactcaaaaaatacgcccggtagtgatcttatttcattatggtgaaagttggaacctcttaggatcctctagatttaagaaggagatatacataaaactccttctgagctagttctctagcattctattattttgattcgacaccttaataatagcagaaggagtttttacctgtcaaagaaccatcaaacccttgatacacaaggctttgacctaattttgaaaaatgatgttgtttctatatagtatcaagataagaaagaaaaggatttttcgctacgctcaaatcctttcccgtcacgggcttctcagggcgttttatggcgggtctgctatgtggtgctatctgactttttgctgttcagcagttcctgccctctgattttccagtctgaccacttcggattatcccgtgacaggtcattcagactggctaatgcacccagtaaggcagcggtatcatcaacggggtctgacgctcagtggaacgaaaactcacgttaagggattttggtcatgagattatcaaaaaggatcttcacctagatccttttaaattaaaaatgaagttttaaatcaatctaaagtatatatgagtaaacttggtctgacagttaccaatgcttaatcagtgaggcacctatctcagcgatctgtctatttcgttcatccatagttgcctgactccccgtcgtgtagataactacgatacgggagggcttaccatctggccccagtgctgcaatgataccgcgagacccacgctcaccggctccagatttatcagcaataaaccagccagccggaagggccgagcgcagaagtggtcctgcaactttatccgcctccatccagtctattaattgttgccgggaagctagagtaagtagttcgccagttaatagtttgcgcaacgttgttgccattgctacaggcatcgtggtgtcacgctcgtcgtttggtatggcttcattcagctccggttcccaacgatcaaggcgagttacatgatcccccatgttgtgcaaaaaagcggttagctccttcggtcctccgatcgttgtcagaagtaagttggccgcagtgttatcactcatggttatggcagcactgcataattctcttactgtcatgccatccgtaagatgcttttctgtgactggtgagtactcaaccaagtcattctgagaatagtgtatgcggcgaccgagttgctcttgcccggcgtcaatacgggataataccgcgccacatagcagaactttaaaagtgctcatcattggaaaacgttcttcggggcgaaaactctcaaggatcttaccgctgttgagatccagttcgatgtaacccactcgtgcacccaactgatcttcagcatcttttactttcaccagcgtttctgggtgagcaaaaacaggaaggcaaaatgccgcaaaaaagggaataagggcgacacggaaatgttgaatactcatactcttcctttttcaatattattgaagcatttatcagggttattgtctcatgagcggatacatatttgaatgtatttagaaaaataaacaaataggggttccgcgcacatttccccgaaaagtgccaccaaaaaaacacaaaagaccacattttttaatgtggtctttattcttcaactaaagcacccattagttcaacaaacgaaaattggataaagtgggatatttttaaaatatatatttatgttacagtaagctgcctcgcgcgtttcggtgatgacggtgaaaacctctgacacatgcagctcccggagacggtcacagcttgtctgtaagcggatgccgggagcagacaagcccgtcagggcgcgtcagcgggtgttggcgggtgtcggggcgcagccatgacccagtcacgtagcgatagcggagtgtatactggcttaactatgcggcatcagagcagattgtactgagagtgcaccatatgcggtgtgaaataccgcacagatgcgtaaggagaaaataccgcatcaggcgctcttccgcttcctcgctcactgactcgctgcgctcggtcgttcggctgcggcgagcggtatcagctcactcaaaggcggtaatacggttatccacagaatcaggggataacgcaggaaagaacatgtgagcaaaaggccagcaaaaggccaggaaccgtaaaaaggccgcgttgctggcgtt

SEQ ID NO: 24 - DNA, 9656 bp, synthetic construct
  source 1..9656: mol_type = other DNA
aaagccatgacaaaaacgcgtaacaaaagtgtctataatcacggcagaaaagtccacattgattatttgcacggcgtcacactttgctatgccatagcatttttatccataagattagcggatcctacctgacgctttttatcgcaactctctactgtttctccatacccgtttttttgggaattcgagctctaaggaggttataaaaaatggatattaatactgaaactgagatcaagcaaaagcattcactaaccccctttcctgttttcctaatcagcccggcatttcgcgggcgatattttcacagctatttcaggagttcagccatgaacgcttattacattcaggatcgtcttgaggctcagagctgggcgcgtcactaccagcagctcgcccgtgaagagaaagaggcagaactggcagacgacatggaaaaaggcctgccccagcacctgtttgaatcgctatgcatcgatcatttgcaacgccacggggccagcaaaaaatccattacccgtgcgtttgatgacgatgttgagtttcaggagcgcatggcagaacacatccggtacatggttgaaaccattgctcaccaccaggttgatattgattcagaggtataaaacgaatgagtactgcactcgcaacgctggctgggaagctggctgaacgtgtcggcatggattctgtcgacccacaggaactgatcaccactcttcgccagacggcatttaaaggtgatgccagcgatgcgcagttcatcgcattactgatcgttgccaaccagtacggccttaatccgtggacgaaagaaatttacgcctttcctgataagcagaatggcatcgttccggtggtgggcgttgatggctggtcccgcatcatcaatgaaaaccagcagtttgatggcatggactttgagcaggacaatgaatcctgtacatgccggatttaccgcaaggaccgtaatcatccgatctgcgttaccgaatggatggatgaatgccgccgcgaaccattcaaaactcgcgaaggcagagaaatcacggggccgtggcagtcgcatcccaaacggatgttacgtcataaagccatgattcagtgtgcccgtctggccttcggatttgctggtatctatgacaaggatgaagccgagcgcattgtcgaaaatactgcatacactgcagaacgtcagccggaacgcgacatcactccggttaacgatgaaaccatgcaggagattaacactctgctgatcgccctggataaaacatgggatgacgacttattgccgctctgttcccagatatttcgccgcgacattcgtgcatcgtcagaactgacacaggccgaagcagtaaaagctcttggattcctgaaacagaaagccgcagagcagaaggtggcagcatgacaccggacattatcctgcagcgtaccgggatcgatgtgagagctgtcgaacagggggatgatgcgtggcacaaattacggctcggcgtcatcaccgcttcagaagttcacaacgtgatagcaaaaccccgctccggaaagaagtggcctgacatgaaaatgtcctacttccacaccctgcttgctgaggtttgcaccggtgtggctccggaagttaacgctaaagcactggcctggggaaaacagtacgagaacgacgccagaaccctgtttgaattcacttccggcgtgaatgttactgaatccccgatcatctatcgcgacgaaagtatgcgtaccgcctgctctcccgatggtttatgcagtgacggcaacggccttgaactgaaatgcccgtttacctcccgggatttcatgaagttccggctcggtggtttcgaggccataaagtcagcttacatggcccaggtgcagtacagcatgtgggtgacgcgaaaaaatgcctggtactttgccaactatgacccgcgtatgaagcgtgaaggcctgcattatgtcgtgattgagcgggatgaaaagtacatggcgagttttgacgagatcgtgccggagttcatcgaaaaaatggacgaggcactggctgaaattggttttgtatttggggagcaatggcgatgagatctaaagaggagaaaggatctatggataagaaatactcaataggcttagatatcggcacaaatagcgtcggatgggcggtgatcactgatgaatataaggttccgtctaaaaagttcaaggttctgggaaatacagaccgccacagtatcaaaaaaaatcttataggggctcttttatttgacagtggagagacagcggaagcgactcgtctcaaacggacagctcgtagaaggtatacacgtcggaagaatcgtatttgttatctacaggagattttttcaaatgagatggcgaaagtagatgatagtttctttcatcgacttgaagagtcttttttggtggaagaagacaagaagcatgaacgtcatcctatttttggaaatatagtagatgaagttgcttatcatgagaaatatccaactatctatcatctgcgaaaaaaattggtagattctactgataaagcggatttgcgcttaatctatttggccttagcgcatatgattaagtttcgtggtcattttttgattgagggagatttaaatcctgataatagtgatgtggacaaactatttatccagttggtacaaacctacaatcaattatttgaagaaaaccctattaacgcaagtggagtagatgctaaagcgattctttctgcacgattgagtaaatcaagacgattagaaaatctcattgctcagctccccggtgagaagaaaaatggcttatttgggaatctcattgctttgtcattgggtttgacccctaattttaaatcaaattttgatttggcagaagatgctaaattacagctttcaaaagatacttacgatgatgatttagataatttattggcgcaaattggagatcaatatgctgatttgtttttggcagctaagaatttatcagatgctattttactttcagatatcctaagagtaaatactgaaataactaaggctcccctatcagcttcaatgattaaacgctacgatgaacatcatcaagacttgactcttttaaaagctttagttcgacaacaacttccagaaaagtataaagaaatcttttttgatcaatcaaaaaacggatatgcaggttatattgatgggggagctagccaagaagaattttataaatttatcaaaccaattttagaaaaaatggatggtactgaggaattattggtgaaactaaatcgtgaagatttgctgcgcaagcaacggacctttgacaacggctctattccccatcaaattcacttgggtgagctgcatgctattttgagaagacaagaagacttttatccatttttaaaagacaatcgtgagaagattgaaaaaatcttgacttttcgaattccttattatgttggtccattggcgcgtggcaatagtcgttttgcatggatgactcggaagtctgaagaaacaattaccccatggaattttgaagaagttgtcgataaaggtgcttcagctcaatcatttattgaacgcatgacaaactttgataaaaatcttccaaatgaaaaagtactaccaaaacatagtttgctttatgagtattttacggtttataacgaattgacaaaggtcaaatatgttactgaaggaatgcgaaaaccagcatttctttcaggtgaacagaagaaagccattgttgatttactcttcaaaacaaatcgaaaagtaaccgttaagcaattaaaagaagattatttcaaaaaaatagaatgttttgatagtgttgaaatttcaggagttgaagatagatttaatgcttcattaggtacctaccatgatttgctaaaaattattaaagataaagattttttggataatgaagaaaatgaagatatcttagaggatattgttttaacattgaccttatttgaagatagggagatgattgaggaaagacttaaaacatatgctcacctctttgatgataaggtgatgaaacagcttaaacgtcgccgttatactggttggggacgtttgtctcgaaaattgattaatggtattagggataagcaatctggcaaaacaatattagattttttgaaatcagatggttttgccaatcgcaattttatgcagctgatccatgatgatagtttgacatttaaagaagacattcaaaaagcacaagtgtctggacaaggcgatagtttacatgaacatattgcaaatttagctggtagccctgctattaaaaaaggtattttacagactgtaaaagttgttgatgaattggtcaaagtaatggggcggcataagccagaaaatatcgttattgaaatggcacgtgaaaatcagacaactcaaaagggccagaaaaattcgcgagagcgtatgaaacgaatcgaagaaggtatcaaagaattaggaagtcagattcttaaagagcatcctgttgaaaatactcaattgcaaaatgaaaagctctatctctattatctccaaaatggaagagacatgtatgtggaccaagaattagatattaatcgtttaagtgattatgatgtcgatcacattgttccacaaagtttccttaaagacgattcaatagacaataaggtcttaacgcgttctgataaaaatcgtggtaaatcggataacgttccaagtgaagaagtagtcaaaaagatgaaaaactattggagacaacttctaaacgccaagttaatcactcaacgtaagtttgataatttaacgaaagctgaacgtggaggtttgagtgaacttgataaagctggttttatcaaacgccaattggttgaaactcgccaaatcactaagcatgtggcacaaattttggatagtcgcatgaatactaaatacgatgaaaatgataaacttattcgagaggttaaagtgattaccttaaaatctaaattagtttctgacttccgaaaagatttccaattctataaagtacgtgagattaacaattaccatcatgcccatgatgcgtatctaaatgccgtcgttggaactgctttgattaagaaatatccaaaacttgaatcggagtttgtctatggtgattataaagtttatgatgttcgtaaaatgattgctaagtctgagcaagaaataggcaaagcaaccgcaaaatatttcttttactctaatatcatgaacttcttcaaaacagaaattacacttgcaaatggagagattcgcaaacgccctctaatcgaaactaatggggaaactggagaaattgtctgggataaagggcgagattttgccacagtgcgcaaagtattgtccatgccccaagtcaatattgtcaagaaaacagaagtacagacaggcggattctccaaggagtcaattttaccaaaaagaaattcggacaagcttattgctcgtaaaaaagactgggatccaaaaaaatatggtggttttgatagtccaacggtagcttattcagtcctagtggttgctaaggtggaaaaagggaaatcgaagaagttaaaatccgttaaagagttactagggatcacaattatggaaagaagttcctttgaaaaaaatccgattgactttttagaagctaaaggatataaggaagttaaaaaagacttaatcattaaactacctaaatatagtctttttgagttagaaaacggtcgtaaacggatgctggctagtgccggagaattacaaaaaggaaatgagctggctctgccaagcaaatatgtgaattttttatatttagctagtcattatgaaaagttgaagggtagtccagaagataacgaacaaaaacaattgtttgtggagcagcataagcattatttagatgagattattgagcaaatcagtgaattttctaagcgtgttattttagcagatgccaatttagataaagttcttagtgcatataacaaacatagagacaaaccaatacgtgaacaagcagaaaatattattcatttatttacgttgacgaatcttggagctcccgctgcttttaaatattttgatacaacaattgatcgtaaacgatatacgtctacaaaagaagttttagatgccactcttatccatcaatccatcactggtctttatgaaacacgcattgatttgagtcagctaggaggtgactaacgcatcctcacgataatatccgggtaggcgcaatcactttcgtctactccgttacaaagcgaggctgggtatttcccggcctttctgttatccgaaatccactgaaagcacagcggctggctgaggagataaataataaacgaggggctgtatgcacaaagcatcttctgttgagttaagaacgagtatcgagatggcacatagccttgctcaaattggaatcaggtttgtgccaataccagtagaaacagacgaagaatccatgggtatggacagttttccctttgatatgtaacggtgaacagttgttctacttttgtttgttagtcttgatgcttcactgatagatacaagagccaaatctagtaatattttatctgattaataagatgatcttcttgagatcgttttggtctgcgcgtaatctcttgctctgaaaacgaaaaaaccgccttgcagggcggtttttcgaaggttctctgagctaccaactctttgaaccgaggtaactggcttggaggagcgcagtcaccaaaacttgtcctttcagtttagccttaaccggcgcatgacttcaagactaactcctctaaatcaattaccagtggctgctgccagtggtgcttttgcatgtctttccgggttggactcaagacgatagttaccggataaggcgcagcggtcggactgaacggggggttcgtgcatacagtccagcttggagcgaactgcctacccggaactgagtgtcaggcgtggaatgagacaaacgcggccataacagcggaatgacaccggtaaaccgaaaggcaggaacaggagagcgcacgagggagccgccagggggaaacgcctggtatctttatagtcctgtcgggtttcgccaccactgatttgagcgtcagatttcgtgatgcttgtcaggggggcggagcctatggaaaaacggctttgccgcggccccgctgaatattccttttgtctccgaccatcaggcacctgagtcgctgtctttttcgtgacattcagttcgctgcgctcacggctctggcagtgaatgggggtaaatggcactacaggcgccttttatggattcatgcaaggaaactacccataatacaagaaaagatgtggtctttattcttcaactaaagcacccattagttcaacaaacgaaaattggataaagtgggatatttttaaaatatatatttatgttacctggcagagcctgtactttttacagtcggttttctaatgtcactaacctgccccgttagtcgccatttgcatcgatttattatgacaacttgacggctacatcattcactttttcttcacaaccggcacggaactcgctcgggctggccccggtgcattttttaaatacccgcgagaaatagagttgatcgtcaaaaccaacattgcgaccgacggtggcgataggcatccgggtggtgctcaaaagcagcttcgcctggctgatacgttggtcctcgcgccagcttaagacgctaatccctaactgctggcggaaaagatgtgacagacgcgacggcgacaagcaaacatgctgtgcgacgctggcgatatcaaaattgctgtctgccaggtgatcgctgatgtactgacaagcctcgcgtacccgattatccatcggtggatggagcgactcgttaatcgcttccatgcgccgcagtaacaattgctcaagcagatttatcgccagcagctccgaatagcgcccttccccttgcccggcgttaatgatttgcccaaacaggtcgctgaaatgcggctggtgcgcttcatccgggcgaaagaaccccgtattggcaaatattgacggccagttaagccattcatgccagtaggcgcgcggacgaaagtaaacccactggtgataccattcgcgagcctccggatgacgaccgtagtgatgaatctctcctggcgggaacagcaaaatatcacccggtcggcaaacaaattctcgtccctgatttttcaccaccccctgaccgcgaatggtgagattgagaatataacctttcattcccagcggtcggtcgataaaaaaatcgagataaccgttggcctcaatcggcgttaaacccgccaccagatgggcattaaacgagtatcccggcagcaggggatcattttgcgcttcagccatacttttcatactcccgccattcagagaagaaaccaattgtccatattgcatcagacattgccgtcactgcgtcttttactggctcttctcgctaaccaaaccggtaaccccgcttattaaaagcattctgtaacaaagcgggaccagtaatagaaagtgagggagccacggttgatgagagctttgttgtaggtggaccagttggtgattttgaacttttgctttgccacggaacggtctgcgttgtcgggaagatgcgtgatctgatccttcaactcagcaaaagttcgatttattcaacaaagccacgttgtgtctcaaaatctctgatgttacattgcacaagataaaaatatatcatcatgaacaataaaactgtctgcttacataaacagtaatacaaggggtgttatgagccatattcaacgggaaacgtcttgctcgaggccgcgattaaattccaacatggatgctgatttatatgggtataaatgggctcgcgataatgtcgggcaatcaggtgcgacaatctatcgattgtatgggaagcccgatgcgccagagttgtttctgaaacatggcaaaggtagcgttgccaatgatgttacagatgagatggtcagactaaactggctgacggaatttatgcctcttccgaccatcaagcattttatccgtactcctgatgatgcatggttactcaccactgcgatccccgggaaaacagcattccaggtattagaagaatatcctgattcaggtgaaaatattgttgatgcgctggcagtgttcctgcgccggttgcattcgattcctgtttgtaattgtccttttaacagcgatcgcgtatttcgtctcgctcaggcgcaatcacgaatgaataacggtttggttgatgcgagtgattttgatgacgagcgtaatggctggcctgttgaacaagtctggaaagaaatgcataagcttttgccattctcaccggattcagtcgtcactcatggtgatttctcacttgataaccttatttttgacgaggggaaattaataggttgtattgatgttggacgagtcggaatcgcagaccgataccaggatcttgccatcctatggaactgcctcggtgagttttctccttcattacagaaacggctttttcaaaaatatggtattgataatcctgatatgaataaattgcagtttcatttgatgctcgatgagtttttctaatcagaattggttaattggttgtaaca